European Patent Application EP 4 789 724 A2, published August 12, 2026. Title: ANTI-4-1BB NANOBODY, PREPARATION THEREFOR, AND USE THEREOF. Applicant: ABLINK BIOTECH CO., LTD. Application WO PCT/CN2023/120848, filed September 22, 2023. The sequence listing filed with the application follows.

SEQUENCE LISTING (28 sequences)

SEQ ID NO: 1 - protein, 116 aa, synthetic construct
QVQLVESGGGLVQPGGSLRLSCVASGFVFSTVTMGWGRQVPGKEFEWVSGVSSEGITDYADSVKGRFTISRDNAKNTVYLEMNSLKSEDTAEYYCLIGGRWSFGTWGQGTQVTVSS

SEQ ID NO: 2 - protein, 123 aa, synthetic construct
QVQLVESGGGLVQPGGSLRLSCAASGFTLDSYAIAWFRQAPGKEREGVSCITSSGGSTNYADSVKGRFTISRDGAKNTVYLQLNSLKPEDTAIYYCAAFHRATCVILGEYDYWGQGTQVTVSS

SEQ ID NO: 3 - protein, 125 aa, synthetic construct
QVQLVESGGGLVHPGGSLRLSCAASGFTLDDSAIGWFRQAPGKEREGVSCRSRSGYMTKYADSVKGRFTISRYNANNTMYLQMNSLKPEDTAVYYCATTRRGYCSGYETKGVDYWGQGIQVTVSS

SEQ ID NO: 4 - protein, 126 aa, synthetic construct
EVQLVESGGGLVQAGASLTLSCVISGRTFSSYAMGWYRQAPGKERAFVGTITWNNDIIYSDSVKGRFTISTDDGKNTMYLQMNNLKPEDTAVYYCAAYSVPYGDFCTLNYDLMDYWGKGTLVTVSS

SEQ ID NO: 5 - protein, 119 aa, synthetic construct
QVQLVESGGGLVHPGGSLRLSCAASGFIFSLYTMSWVRQAPGKGLEWVSDINSGGDSTDYADSVKGRFTISRDNAKSTLYLQMNSLKPEDTAVYYCAKDYPLGQREDYWGQGTQVTVSS

SEQ ID NO: 6 - protein, 130 aa, synthetic construct
QVQLVESGGGLVQTGGSLTLSCVASGRRFEAYTIGWLRQAPGDLREGVGCIFGGTTFTGYDDSVKGRFTISRDTAKNTVYLRMNNLTSEDTATYYCAAEGRPGQIKGQHGCLTPSWYNYKGQGTQVTVSS

SEQ ID NO: 7 - protein, 124 aa, synthetic construct
QVQLVESGGGLVHVGESLTLSCVISGGSSNLYGIGWYRQAPGQERKLVAVLHNEHTTKYLDSVKGRFFVSGDNAKNTLYLHMNNVKVEDTAVYYCNSASGTLAGTGYFASVGPWGQGTLVTVSS

SEQ ID NO: 8 - protein, 5 aa, synthetic construct
TVTMG

SEQ ID NO: 9 - protein, 16 aa, synthetic construct
GVSSEGITDYADSVKG

SEQ ID NO: 10 - protein, 8 aa, synthetic construct
GGRWSFGT

SEQ ID NO: 11 - protein, 5 aa, synthetic construct
SYAIA

SEQ ID NO: 12 - protein, 17 aa, synthetic construct
CITSSGGSTNYADSVKG

SEQ ID NO: 13 - protein, 14 aa, synthetic construct
FHRATCVILGEYDY

SEQ ID NO: 14 - protein, 5 aa, synthetic construct
DSAIG

SEQ ID NO: 15 - protein, 17 aa, synthetic construct
CRSRSGYMTKYADSVKG

SEQ ID NO: 16 - protein, 16 aa, synthetic construct
TRRGYCSGYETKGVDY

SEQ ID NO: 17 - protein, 5 aa, synthetic construct
SYAMG

SEQ ID NO: 18 - protein, 16 aa, synthetic construct
TITWNNDIIYSDSVKG

SEQ ID NO: 19 - protein, 18 aa, synthetic construct
YSVPYGDFCTLNYDLMDY

SEQ ID NO: 20 - protein, 5 aa, synthetic construct
LYTMS

SEQ ID NO: 21 - protein, 17 aa, synthetic construct
DINSGGDSTDYADSVKG

SEQ ID NO: 22 - protein, 10 aa, synthetic construct
DYPLGQREDY

SEQ ID NO: 23 - protein, 5 aa, synthetic construct
AYTIG

SEQ ID NO: 24 - protein, 17 aa, synthetic construct
CIFGGTTFTGYDDSVKG

SEQ ID NO: 25 - protein, 21 aa, synthetic construct
EGRPGQIKGQHGCLTPSWYNY

SEQ ID NO: 26 - protein, 5 aa, synthetic construct
LYGIG

SEQ ID NO: 27 - protein, 16 aa, synthetic construct
VLHNEHTTKYLDSVKG

SEQ ID NO: 28 - protein, 16 aa, synthetic construct
ASGTLAGTGYFASVGP